European Patent Application EP 4 345 166 A2, published April 3, 2024. Title: METHOD FOR PRODUCING L-AMINO ACID. Applicant: 味の素株式会社. The sequence listing filed with the application follows.

SEQUENCE LISTING (20 sequences)

SEQ ID NO: 1 - DNA, 768 bp, Pantoea ananatis
  source 1..768: mol_type = genomic DNA
atgcgggttgcgcttgtgacaggtgcgggtcagggcattggtgaggcgatagccttacgtctggcaaaagacggatttgccgtggccgtggctgattacaatattgaaaccgcgtcgcaggttgcggaaaagatcaagaaagatggcggccgtgcgctggccatcaaggtggatgtaacaaaacgggatcaggtatttcatgccgttgaagaagcgcgcagcgtattgggtgattttaacgtcattgtgaataacgcaggtgtcgcgccctcaacgcccattgatgaaatcaccgaagaggtcatcaacaaggtttacgacgttaatgtcaaaggcgtgatctggggcatgcaggcagcaataaaagcgttcgcgtctgaaggtcatggcggaaaaattattaacgcctgttctcaggccgggcatgtcggcaatcccgagctggcagtttacagctcaagcaagtttgctgttcggggcctgacacaaactgccgcacgggatctggcaccggcggggatcaccgtgaatggcttttgtcctggtattgttaaaacaccgatgtgggcggagatcgacaggcagatttccgaagcggcaggcaaacccgtgggttatggtactcaggagtttgcgaaaagaatcacgcttggtcggttatcagaacccgaagatgtcgcagcctgtgtcgcctttcttgccggcccggattctgattacatcaccggacagtcgttactggtagacggtggcatggtgtttagctaa

SEQ ID NO: 2 - protein, 255 aa, Pantoea ananatis
MRVALVTGAGQGIGEAIALRLAKDGFAVAVADYNIETASQVAEKIKKDGGRALAIKVDVTKRDQVFHAVEEARSVLGDFNVIVNNAGVAPSTPIDEITEEVINKVYDVNVKGVIWGMQAAIKAFASEGHGGKIINACSQAGHVGNPELAVYSSSKFAVRGLTQTAARDLAPAGITVNGFCPGIVKTPMWAEIDRQISEAAGKPVGYGTQEFAKRITLGRLSEPEDVAACVAFLAGPDSDYITGQSLLVDGGMVFS

SEQ ID NO: 3 - DNA, 1680 bp, Pantoea ananatis
  source 1..1680: mol_type = genomic DNA
atgaaaactatctctgatacgacactctggcactgcggtgcagacctggttgtcgcgcaacttgaagcgcaaggcgtcagccatgtgtttggcatccctggcgcaaaaattgataaggtatttgattccctactcgattcttccattcagacgatccccgtgcggcatgaggcgaatgccgcctttatggccgcggcagtaggccgtctgacgggtaacgctggcgtggcgctggtcacatccgggccgggctgctcaaacctggtgaccggtatggctaccgcaaccagtgagggcgacccggtggtggctattgggggcgcggtcaaacgctccgacagcgccaagcaggttcaccagagtcttgataccgtatccatgttccgcccggtgacaaaatatgcggttgaagtcaccgactcgtcggcactggcggaatgtgtatcaaacgcgtttcgtcacgctgaacacggtcgcggcggcggtgcgtttgtcagcctgccacaggatatcgttgatcagccggtcacgggtaaggtgctgagccatcacggccgcatcacgctgggtgcggcaccggatgtgatgattgatgcggtcagtcgcgagatcgcccacgcaaaaaatcccgtgatcttgctgggcctgatggcaagccagcctgagaatagcgaagccattcacgatctgttaaaccgcagccatatcccggtaaccagcacgtatcaggcggcgggtgccgttcgccaggagcacttttcccgttttgccggtcgcgtgggacttttcaacaatcaggcaggcgacaagctgctgcaacaggccgacctgattattaccatcggctacagcccggttgagtatgaacctgccatgtggaacagcgggaatgccaccttaatccacattgacgttgtgccagcggaaacggacaaccgctatttgccagatgcggagctggtcggcaacatcgccgccacgctgcgtaaactggcacaaaaggtcagccagccgttacagctcagcaaggaggctgccagtatccttgaggaccgtcagcagcagcggcagttacttgcattacagggcgcgagcctgaatcagtttgctcttcatccgctgcgcatcgtgcgtgcgatgcaggacattatcaacagcgacgtcagcctcaccgttgatatgggcagcttccatatctggattgcccgctatctctacagcttccgcgcacgccaaatcatgatttctaacgggcagcaaaccatgggcgtggccttgccctgggcgattggtgcctggctggtcgatccacagcgtaaagtcgtctcggtttcaggagatggcggcttcatgcagtcaagcatggagctggaaaccgccgtcaggctcaacgccaacattttacacattgtctgggtcgataatgcttacaacatggtggcgatgcaggaagagaaaaaatatcagcgtgtttcaggcgtgaactttgggcccattgattttaaagcctatgcggaagcattcggtgcggcgggattcgcggtgaacagtgcctccgaactggaacccacgctgcgcaaagcgatggatgttcaggggcctgctgttgtggcagtgccagtggattacgccgataaccacttgctgatggggcagcttcatctcagccagttactttaa

SEQ ID NO: 4 - protein, 559 aa, Pantoea ananatis
MKTISDTTLWHCGADLVVAQLEAQGVSHVFGIPGAKIDKVFDSLLDSSIQTIPVRHEANAAFMAAAVGRLTGNAGVALVTSGPGCSNLVTGMATATSEGDPVVAIGGAVKRSDSAKQVHQSLDTVSMFRPVTKYAVEVTDSSALAECVSNAFRHAEHGRGGGAFVSLPQDIVDQPVTGKVLSHHGRITLGAAPDVMIDAVSREIAHAKNPVILLGLMASQPENSEAIHDLLNRSHIPVTSTYQAAGAVRQEHFSRFAGRVGLFNNQAGDKLLQQADLIITIGYSPVEYEPAMWNSGNATLIHIDVVPAETDNRYLPDAELVGNIAATLRKLAQKVSQPLQLSKEAASILEDRQQQRQLLALQGASLNQFALHPLRIVRAMQDIINSDVSLTVDMGSFHIWIARYLYSFRARQIMISNGQQTMGVALPWAIGAWLVDPQRKVVSVSGDGGFMQSSMELETAVRLNANILHIVWVDNAYNMVAMQEEKKYQRVSGVNFGPIDFKAYAEAFGAAGFAVNSASELEPTLRKAMDVQGPAVVAVPVDYADNHLLMGQLHLSQLL

SEQ ID NO: 5 - DNA, 783 bp, Pantoea ananatis
  source 1..783: mol_type = genomic DNA
atgagcaattttgtaactgattgttcctgcgaggatcaactaaaagataccgtccaaaagctgcgaaaaaacatgccagaaagtgttatgtatcaaacctctttgatgagtgcgctgctgagtggtgtttatgacggtgaaaccaggattgctgacttactgcgcaaaggtgactttggtctgggaaccttcaatcagctggatggtgaactcattgcgttcgacagcaatgtgtatcagctgcgcgccgatggcagtgcccggcctgctgatcctgaccagaaaacgccatttgcggtaatgaccttttttcaaccccagcataaacacgtttttgaacgcgcggttcagcgcgatgcgctgcaccagcttatcgacagcgaaatcacctccgacaaccagttttgtgcactgcgtgtaagcggacatttttcatccgtccagacgcgtaccgttccgtgccagtgccggccttaccgatcgatgcctgaagttctgggaaaccagcccatatttgaattcacgcatcgccatggcgagcttattggcttccgcacgccgcagtacatgcagggtatcaacgtcgcaggatatcacgaacatttcatcacagacgacagaaccggcggtgggcatatcctggattatgtgctggagcagggcacgctgacttttggtgccatcagcaagctggtgatcgatttacctgaaaacgccgactttcttaatgccaacctgacgccggaaaacctggatgatgccatccgttctgtcgaaagctaa

SEQ ID NO: 6 - protein, 260 aa, Pantoea ananatis
MSNFVTDCSCEDQLKDTVQKLRKNMPESVMYQTSLMSALLSGVYDGETRIADLLRKGDFGLGTFNQLDGELIAFDSNVYQLRADGSARPADPDQKTPFAVMTFFQPQHKHVFERAVQRDALHQLIDSEITSDNQFCALRVSGHFSSVQTRTVPCQCRPYRSMPEVLGNQPIFEFTHRHGELIGFRTPQYMQGINVAGYHEHFITDDRTGGGHILDYVLEQGTLTFGAISKLVIDLPENADFLNANLTPENLDDAIRSVES

SEQ ID NO: 7 - DNA, 726 bp, Pantoea ananatis
  source 1..726: mol_type = genomic DNA
atgtcagaccagaaaaagggtcattcacgcagggattttttgctgaagaccatcaccctggcgcccgcagtggcggtaggcagtagcgcacttggtgcattttctgcgcccgctcaggcggcagcgcccgccgcaccccagcccgcccgagattatcagcccacttggtttaccgccgaggaatttgcctttatcaaggcggccgttgcgcgcctgattcctgctgatgaacgcggccccggcgcgctggaagcaggcgtgcctgagtttatcgatcgtcagatgaatatgccttacgccaccggagcgaactggtatatgcaggggcctttcaatcccgacgtccctaaagaaatgggctatcagctgccgctggtgccgcaacagatctaccgtctcggtctggctgatgccgatcattacagtcagcagcagcacggtaaggtgtttgcccaactcgacgccgggcagcaggacgcattattacaggccatggagagcggcaaagccggtttccgtcagctgcccgccaacgtgtttttctcatacttattgcagaacacccgcgaaggcttctttagcgatcccatccacggcggcaatcagggcatggtgggctggaagctcatcaacttccctggcgcacgcgccgactttatggactgggtagagcgcggtgaacgctatccgttcccgtcagtgtcgattcgtggagagagaagctga

SEQ ID NO: 8 - protein, 241 aa, Pantoea ananatis
MSDQKKGHSRRDFLLKTITLAPAVAVGSSALGAFSAPAQAAAPAAPQPARDYQPTWFTAEEFAFIKAAVARLIPADERGPGALEAGVPEFIDRQMNMPYATGANWYMQGPFNPDVPKEMGYQLPLVPQQIYRLGLADADHYSQQQHGKVFAQLDAGQQDALLQAMESGKAGFRQLPANVFFSYLLQNTREGFFSDPIHGGNQGMVGWKLINFPGARADFMDWVERGERYPFPSVSIRGERS

SEQ ID NO: 9 - DNA, 1785 bp, Pantoea ananatis
  source 1..1785: mol_type = genomic DNA
atggcaaatgaattaaagaaagtggatgccgtgattgtcggctttggctgggcgggcgccattatggccaaagagctgaccgaagcaggtctgaacgtgctggcgctggagcgcggtccacatcgtgatacctatccggatggttcttacccgcagtcgattgatgagctgacctacaacgttcgcaaaaagctgtttcaggacctgtctaagagcaccgtcaccattcggcacgacgcctcacaaacggccgtgccttaccgccaactggcggccttcctgcccggtaccggtaccggcggcgccgggctgcactggtcgggtgtccatttccgggttgatcccgtagagctgaagctgcgtagccactatgaggcgcgctacggtaaaaactttattcctgaaggcatgaccattcaggactttggcgtggactaccaggagctggagccgttttttgataaagctgaaaaggtgtttggcacctccggtagtgcctggagtattcagggcaaggtcgtcggcaaagacaaaggcggtaacccctttgcgcccgatcgctctgacaactttccactgcccgcgcaaaagcgtacctggtcggctcagctgttcgcccaggccgccgagtccgtaggttatcacccttacgatctgccgtcggcgaacacctctggcccctataccaatacttacggcgcccagatggggccgtgcaacttctgcggctactgcagcggctacgcctgttatatgtattccaaggcatcgccgaatgtgaatattttgcctgcgctgcgtcaggagccaaagtttgagctgcgtaacaattcttacgtgctgcgcgtcaacctcacgggtgataagcagcgtgcgaccggtgtcacctatgtcgatgcgcagggccgtgagcaggtgcaaccggcggatctggtcattctgtctgcctttcagttccataacgtccatttgatgctgttgtccggcattggtaaaccttacaacccgatcaccaacgaagggacgatagggcgcaacttcgcctatcaaaacctgtcgacgttgaaagcgctgttcgataaaaacaccaccaccaatcccttcatcggtgcaggcggtgcaggcgtcgccgtggatgatttcaatgctgacaatttcgatcatggtccgcacggctttgttggcgggtcgccgttctgggtgaaccaggcgggcaccaaaccgatctcggggctccccacgccgaccggcacgccaaactggggcagtcagtggaaagccgccgtggcggacacctacacgcaccacctttccatggatgctcacggtgcgcaccagtcttaccgcgctaactatctggacctggacccgaactacaaagatgcctacggccagccgttgctgcgcatgacgttcgactggcaggacaacgacatcaaaatggcgcagttcatggtggggaaaatgcataaaatcgccgaagccatgaatcctaaaatgatcattggcggggcgaagaagcctggtacgcattttgacacgaccgtgtatcagacgacccacatcagcggcggcgcgattatgggtgaagatcccaataccagtgcggtgaaccgctatctgcaaagctgggatgtgccgaatgtgttcgttcccggcgcttcagcgtttccgcaggggctgggatataaccccaccggcatggtcgccgcactgacctactggtcggcgaaagcgattcgggaacagtatctgaagaatccgggtcccctggtgcaggcataa

SEQ ID NO: 10 - protein, 594 aa, Pantoea ananatis
MANELKKVDAVIVGFGWAGAIMAKELTEAGLNVLALERGPHRDTYPDGSYPQSIDELTYNVRKKLFQDLSKSTVTIRHDASQTAVPYRQLAAFLPGTGTGGAGLHWSGVHFRVDPVELKLRSHYEARYGKNFIPEGMTIQDFGVDYQELEPFFDKAEKVFGTSGSAWSIQGKVVGKDKGGNPFAPDRSDNFPLPAQKRTWSAQLFAQAAESVGYHPYDLPSANTSGPYTNTYGAQMGPCNFCGYCSGYACYMYSKASPNVNILPALRQEPKFELRNNSYVLRVNLTGDKQRATGVTYVDAQGREQVQPADLVILSAFQFHNVHLMLLSGIGKPYNPITNEGTIGRNFAYQNLSTLKALFDKNTTTNPFIGAGGAGVAVDDFNADNFDHGPHGFVGGSPFWVNQAGTKPISGLPTPTGTPNWGSQWKAAVADTYTHHLSMDAHGAHQSYRANYLDLDPNYKDAYGQPLLRMTFDWQDNDIKMAQFMVGKMHKIAEAMNPKMIIGGAKKPGTHFDTTVYQTTHISGGAIMGEDPNTSAVNRYLQSWDVPNVFVPGASAFPQGLGYNPTGMVAALTYWSAKAIREQYLKNPGPLVQA

SEQ ID NO: 11 - DNA, 1317 bp, Pantoea ananatis
  source 1..1317: mol_type = genomic DNA
atggtgatgaaaaacggtattttagccctggtgttgggcagcctcgccttcgccgccctggcggatgacagcacggcggatcgggtcaaacgcggtgaatatctggcgcgcgcgggcgactgtgtagcctgccacagcagtgaaggcggcaagccctttgcagggggattgccgatggccacgccgattggcacgatctactccaccaatatcacgccggataaatcgaccggtattggtgactacagctacgacgactttcagaaagccgtgcggcacggtatcgcgaaaaacggcgatacgctctatcccgctatgccttatccgtcttatgccgtggtcagcgatgaagacatgcaggcgctgtatgcctacttcatgcacggagttgccccggtcagtcaggccaacaaagagagtgatattccctggcccctgtcaatgcgctggccgctggcgatctggcgcaacctgtttgcaccggatgtaaaggcgttccagcctgccgcgcaggaggatgcgacgctggcgcgtggccgctacctggtagaaggtctgggccactgcggtgcctgccatacgccgcgtagttttaccctgcaggaaaaggcgttaaccaatgccgggggaacggattatctggcgggcagcagtgcgccggttgacggctggaccgcaagcaatttgcgcggagataaccgcgatggcttgggccgctggagtgaagatgacctgcgccagttcctgcgctatgggcgtaacgaccacacggcggcatttggcggcatggtggacgttgtcgaccacagcctgcagcacctgacggatgaagacatcacggccatcgcccgctatctgaagtcgctgggtgccaaagatccgcatcaggtggcgtttagcgtggatgacgcgacggccaaagccttatggaagggcgacgacagtcagacgggcgccgcgacctatgtggacagctgcgcagcctgccataaaaccgatggcagcggctataaacgcttctatcctgcgctgcggggcaatcctgtggtgatggcagacgatccgacctcgctgattcacatcgtgctggttggtggcgaactgcgtggagtaaaaggcgcgccttcaaccatcactatgccggcatttggctggcgtctgaacgatcagcaggtcgcggacgtggtgaactttattcgtcgcagctggggcaacaatgcggcggataacgtgacggcgaagcaggtggctgccctgcgtgaagaggtcaaagatcgtcagggcaatgcagatatcaaggtgttagaagggaagtag

SEQ ID NO: 12 - protein, 438 aa, Pantoea ananatis
MVMKNGILALVLGSLAFAALADDSTADRVKRGEYLARAGDCVACHSSEGGKPFAGGLPMATPIGTIYSTNITPDKSTGIGDYSYDDFQKAVRHGIAKNGDTLYPAMPYPSYAVVSDEDMQALYAYFMHGVAPVSQANKESDIPWPLSMRWPLAIWRNLFAPDVKAFQPAAQEDATLARGRYLVEGLGHCGACHTPRSFTLQEKALTNAGGTDYLAGSSAPVDGWTASNLRGDNRDGLGRWSEDDLRQFLRYGRNDHTAAFGGMVDVVDHSLQHLTDEDITAIARYLKSLGAKDPHQVAFSVDDATAKALWKGDDSQTGAATYVDSCAACHKTDGSGYKRFYPALRGNPVVMADDPTSLIHIVLVGGELRGVKGAPSTITMPAFGWRLNDQQVADVVNFIRRSWGNNAADNVTAKQVAALREEVKDRQGNADIKVLEGK

SEQ ID NO: 13 - DNA, 74 bp, synthetic construct
  source 1..74: mol_type = other DNA
  misc_feature 1..74: note = primer
ttagctaaacaccatgccaccgtctaccagtaacgactgtccggtgatgtaatcagtgaagcctgcttttttat

SEQ ID NO: 14 - DNA, 69 bp, synthetic construct
  source 1..69: mol_type = other DNA
  misc_feature 1..69: note = primer
atgagcaattttgtaactgattgttcctgcgaggatcaactaaaagatacccgctcaagttagtataaa

SEQ ID NO: 15 - DNA, 20 bp, synthetic construct
  source 1..20: mol_type = other DNA
  misc_feature 1..20: note = primer
ctacctcatgcgaggtgaca

SEQ ID NO: 16 - DNA, 20 bp, synthetic construct
  source 1..20: mol_type = other DNA
  misc_feature 1..20: note = primer
aacgtagatggcgcagttcc

SEQ ID NO: 17 - DNA, 81 bp, synthetic construct
  source 1..81: mol_type = other DNA
  misc_feature 1..81: note = primer
accactacaacgcactcacttctctttttcgtaccgcagttgatgcggtgatgaggcaatgtctgaagcctgcttttttat

SEQ ID NO: 18 - DNA, 80 bp, synthetic construct
  source 1..80: mol_type = other DNA
  misc_feature 1..80: note = primer
caggctggaacatatctgaacattcagccttccccctgcggggaaggctgaaacactgaggtcgctcaagttagtataaa

SEQ ID NO: 19 - DNA, 20 bp, synthetic construct
  source 1..20: mol_type = other DNA
  misc_feature 1..20: note = primer
ggatggttgtcagttagtcg

SEQ ID NO: 20 - DNA, 20 bp, synthetic construct
  source 1..20: mol_type = other DNA
  misc_feature 1..20: note = primer
gctgagtatgctgatggtga